European Patent Specification EP 3 950 958 B1, published October 4, 2023. Title: Sequencing algorithm. Applicant: Longas Technologies Pty Ltd. The sequence listing filed with the application follows.

SEQUENCE LISTING (291 sequences)

SEQ ID NO: 1 - DNA, 2325 bp, Thermococcus sp. KS-1
atgatcctcgacactgactacataactgagaatggaaaacccgtcataaggattttcaagaaggagaacggcgagtttaagattgagtacgataggacttttgaaccctacatttacgccctcctgaaggacgattctgccattgaggaggtcaagaagataaccgccgagaggcacggaacggttgtaacggttaagcgggctgaaaaggttcagaagaagttcctcgggagaccagttgaggtctggaaactctactttactcaccctcaggacgtcccagcgataagggacaagatacgagagcatccagcagttattgacatctacgagtacgacatacccttcgccaagcgctacctcatagacaagggattagtgccaatggaaggcgacgaggagctgaaaatgcttgcctttgatatcgagacgctctaccatgagggcgaggagttcgccgaggggccaatccttatgataagctacgccgacgaggaaggggccagggtgataacgtggaagaacgcggatctgccctacgttgacgtcgtctcgacggagagggagatgataaagcgcttcctaaaggtggtcaaagagaaagatcctgacgtcctaataacctacaacggcgacaacttcgacttcgcctacctaaaaaaacgctgtgaaaagcttggaataaacttcacgctcggaagggacggaagcgagccgaagattcagaggatgggcgacaggtttgccgtcgaagtgaagggacggatacacttcgatctctatcctgtgataagacggacgataaacctgcccacatacacgcttgaggccgtttatgaagccgtcttcggtcagccgaaggagaaggtctacgctgaggagatagctacagcttgggagagcggtgaaggccttgagagagtagccagatactcgatggaagatgcgaaggtcacatacgagcttgggaaggagtttttccctatggaggcccagctttctcgcttaatcggccagtccctctgggacgtctcccgctccagcactggcaacctcgttgagtggttcctcctcaggaaggcctacgagaggaatgagctggccccgaacaagcccgatgaaaaggagctggccagaagacgacagagctatgaaggaggctatgtaaaagagcccgagagagggttgtgggagaacatagtgtacctagattttagatctctgtacccctcaatcatcatcacccacaacgtctcgccggatactctcaacagggaaggatgcaaggaatatgacgttgccccccaggtcggtcaccgcttctgcaaggacttcccaggatttatcccgagcctgcttggagacctcctagaggagaggcagaagataaagaagaagatgaaggccacgattgacccgatcgagaggaagctcctcgattacaggcagagggccatcaagatcctggccaacagctactacggttactacggctatgcaagggcgcgctggtactgcaaggagtgtgcagagagcgtaacggcctggggaagggagtacataacgatgaccatcagagagatagaggaaaagtacggctttaaggtaatctacagcgacaccgacggattttttgccacaatacctggagccgatgctgaaaccgtcaaaaagaaggcgatggagttcctcaagtatatcaacgccaaactcccgggcgcgcttgagctcgagtacgagggcttctacaaacgcggcttcttcgtcacgaagaagaagtacgcggtgatagacgaggaaggcaagataacaacgcgcggacttgagattgtgaggcgcgactggagcgagatagcgaaagagacgcaggcgagggttcttgaagctttgctaaaggacggtgacgtcgagaaggccgtgaggatagtcaaagaagttaccgaaaagctgagcaagtacgaggttccgccggagaagctggtgatccacgagcagataacgagggatttaaaggactacaaggcaaccggtccccacgttgccgttgccaagaggttggccgcgagaggagtcaaaatacgccctggaacggtgataagctacatcgtgctcaagggctctgggaggataggcgacagggcgataccgttcgacgagttcgacccgacgaagcacaagtacgacgccgagtactacattgagaaccaggttctcccagccgttgagagaattctgagagccttcggttaccgcaaggaagacctgcgctaccagaagacgagacaggttggtctgggagcctggctgaagccgaagggaacttga

SEQ ID NO: 2 - protein, 774 aa, Thermococcus sp. KS-1
MILDTDYITENGKPVIRIFKKENGEFKIEYDRTFEPYIYALLKDDSAIEEVKKITAERHGTVVTVKRAEKVQKKFLGRPVEVWKLYFTHPQDVPAIRDKIREHPAVIDIYEYDIPFAKRYLIDKGLVPMEGDEELKMLAFDIETLYHEGEEFAEGPILMISYADEEGARVITWKNADLPYVDVVSTEREMIKRFLKVVKEKDPDVLITYNGDNFDFAYLKKRCEKLGINFTLGRDGSEPKIQRMGDRFAVEVKGRIHFDLYPVIRRTINLPTYTLEAVYEAVFGQPKEKVYAEEIATAWESGEGLERVARYSMEDAKVTYELGKEFFPMEAQLSRLIGQSLWDVSRSSTGNLVEWFLLRKAYERNELAPNKPDEKELARRRQSYEGGYVKEPERGLWENIVYLDFRSLYPSIIITHNVSPDTLNREGCKEYDVAPQVGHRFCKDFPGFIPSLLGDLLEERQKIKKKMKATIDPIERKLLDYRQRAIKILANSYYGYYGYARARWYCKECAESVTAWGREYITMTIREIEEKYGFKVIYSDTDGFFATIPGADAETVKKKAMEFLKYINAKLPGALELEYEGFYKRGFFVTKKKYAVIDEEGKITTRGLEIVRRDWSEIAKETQARVLEALLKDGDVEKAVRIVKEVTEKLSKYEVPPEKLVIHEQITRDLKDYKATGPHVAVAKRLAARGVKIRPGTVISYIVLKGSGRIGDRAIPFDEFDPTKHKYDAEYYIENQVLPAVERILRAFGYRKEDLRYQKTRQVGLGAWLKPKGT

SEQ ID NO: 3 - DNA, 2325 bp, Thermococcus celer
atgatcctcgacgctgactacatcaccgaagatgggaagcccgtcgtgaggatattcaggaaggagaagggcgagttcagaatcgactacgacagggacttcgagccctacatctacgccctcctgaaggacgattcggccatcgaggaggtgaagaggataaccgttgagcgccacgggaaggccgtcagggttaagcgggtggagaaggtcgaaaagaagttcctcaacaggccgatagaggtctggaagctctacttcaatcacccgcaggacgttccggcgataagggacgagataaggaagcatccggccgtcgttgatatctacgagtacgacatccccttcgccaagcgctacctcatcgataaggggctcgtcccgatggagggggaggaggagctcaaactgatggccttcgacatcgagaccctctaccacgagggagacgagttcggggaggggccgatcctgatgataagctacgccgacggggacggggcgagggtcataacctggaagaagatcgacctcccctacgtcgacgtcgtctcgaccgagaaggagatgataaagcgcttcctccaggtggtgaaggagaaggacccggacgtgctcgtaacttacaacggcgacaacttcgacttcgcctacctgaagagacgctccgaggagcttggattgaagttcatcctcgggagggacgggagcgagcccaagatccagcgcatgggcgaccgcttcgccgtcgaggtgaaggggaggatacacttcgacctctacccggtgataaggcgcaccgtgaacctgccgacctacacgctcgaggcggtctacgaggccatcttcgggaggccaaaggagaaggtctacgccggggagatagtggaggcctgggaaaccggcgagggtcttgagagggttgcccgctactccatggaggacgcaaaggttaccttcgagctcgggagggagttcttcccgatggaggcccagctctcgaggctcatcggccagggtctctgggacgtctcccgctcgagcaccggcaacctggtcgagtggttcctcctgaggaaggcctacgagaggaacgaactggccccgaacaagccgagcggccgggaagtggagatcaggaggcgtggctacgccggtggttacgttaaggagccggagaggggtttatgggagaacatcgtgtacctcgactttcgctctctttacccctccatcatcataacccacaacgtctcgcccgataccctaaacagggagggctgtgagaactacgacgtcgccccccaggtggggcataagttctgcaaagattttccgggcttcatcccgagcctgctcggaggcctgcttgaggagaggcagaagataaagcggaggatgaaggcctctgtggatcccgttgagcggaagctcctcgattacaggcagagggccatcaagatactggccaacagcttctacggatactacggctacgcgagggcgaggtggtactgcagggagtgcgcggagagcgttaccgcctggggcagggagtacatcgatagggtcatcagggagctcgaggagaagttcggcttcaaggtgctctacgcggacacggacggactgcacgccacgatccccggggcggacgccgggaccgtcaaggagagggcgagggggttcctgagatacatcaaccccaagctccccggcctcctggagctcgagtacgaggggttctacctgaggggtttcttcgtgacgaagaagaagtacgcggtcatagacgaggagggcaagataaccacgcgcggcctcgagatagtcaggcgggactggagcgaggtggccaaggagacgcaggcgagggtcctggaggcgatactgaggcacggtgacgtcgaggaggccgttagaatcgtcagggaggtaaccgaaaagctgagcaagtacgaggttccgccggagaaactggtgatccacgagcagataacgagggatttgagggactacaaagccacgggaccgcacgtggcggtggcgaagcgcctggccgggaggggggtaaggatacgccccgggacggtgataagctacatcgtcctcaagggctccggaaggataggggacagggcgattcccttcgacgagttcgacccgactaagcacaggtacgacgccgactactacatcgagaaccaggttctgccagccgtcgagaggatcctgaaggccttcggctaccgcaaggaggacctgaaataccagaagacgaggcaggtgggcctgggtgcgtggctcaacgcggggaaggggtga

SEQ ID NO: 4 - protein, 774 aa, Thermococcus celer
MILDADYITEDGKPVVRIFRKEKGEFRIDYDRDFEPYIYALLKDDSAIEEVKRITVERHGKAVRVKRVEKVEKKFLNRPIEVWKLYFNHPQDVPAIRDEIRKHPAVVDIYEYDIPFAKRYLIDKGLVPMEGEEELKLMAFDIETLYHEGDEFGEGPILMISYADGDGARVITWKKIDLPYVDVVSTEKEMIKRFLQVVKEKDPDVLVTYNGDNFDFAYLKRRSEELGLKFILGRDGSEPKIQRMGDRFAVEVKGRIHFDLYPVIRRTVNLPTYTLEAVYEAIFGRPKEKVYAGEIVEAWETGEGLERVARYSMEDAKVTFELGREFFPMEAQLSRLIGQGLWDVSRSSTGNLVEWFLLRKAYERNELAPNKPSGREVEIRRRGYAGGYVKEPERGLWENIVYLDFRSLYPSIIITHNVSPDTLNREGCENYDVAPQVGHKFCKDFPGFIPSLLGGLLEERQKIKRRMKASVDPVERKLLDYRQRAIKILANSFYGYYGYARARWYCRECAESVTAWGREYIDRVIRELEEKFGFKVLYADTDGLHATIPGADAGTVKERARGFLRYINPKLPGLLELEYEGFYLRGFFVTKKKYAVIDEEGKITTRGLEIVRRDWSEVAKETQARVLEAILRHGDVEEAVRIVREVTEKLSKYEVPPEKLVIHEQITRDLRDYKATGPHVAVAKRLAGRGVRIRPGTVISYIVLKGSGRIGDRAIPFDEFDPTKHRYDADYYIENQVLPAVERILKAFGYRKEDLKYQKTRQVGLGAWLNAGKG

SEQ ID NO: 5 - DNA, 2328 bp, Thermococcus siculi
atgatcctcgacacggactacatcacggaagatgggaaacccgtcataaggatattcaagaaagagaacggcgagttcaagatcgagtacgacaggacttttgaaccctacatctacgccctcctgaaggacgactccgcgattgaggatgttaaaaagataaccgccgagaggcacggaacggtggtgaaggtcaagcgcgccgaaaaggtgcagaagaagttcctaggcaggccggttgaagtctggaagctctacttcacccacccccaagatgtcccggcgataagggacaagattaggaagcatccagctgtaattgacatctacgagtacgacataccattcgccaagcgctacctcatcgacaagggcctgattccgatggagggtgaagaagagcttaagatgctcgccttcgacattgagacgctctaccatgagggtgaggagttcgccgaggggcctattctgatgataagctacgccgacgagagcgaggcacgcgtcatcacctggaagaaaatcgacctcccctacgttgacgtcgtctcaacggagaaggagatgataaagcgcttcctccgcgttgtgaaggagaaagatcccgatgtcctcataacctacaacggcgacaacttcgacttcgcctacctgaagaagcgctgtgaaaagcttggaataaacttcctccttggaagggacgggagcgagccgaagatccagagaatgggtgaccgcttcgccgttgaggtgaaggggaggatacacttcgacctctatcctgtaataaggcgcacgataaacctgccgacctacatgcttgaggcagtctacgaggccatctttgggaagccaaaggagaaggtttacgccgaggagatagccaccgcttgggaaaccggagagggccttgagagggtggctcgctactctatggaggacgcgaaggtcacgtttgagcttggaaaggagttcttcccgatggaggcccaactttcgaggttggtcggccagagcttctgggatgtcgcgcgctcaagcacgggcaatctggtcgagtggttcctcctcaggaaggcctacgagaggaacgagctggctccaaacaagccctctggaagggaatatgacgagaggcgcggtggatacgccggcggctacgtcaaggaaccggaaaagggcctgtgggagaacatagtctacctcgactataaatctctctacccctcaatcatcatcacccacaacgtctcgcccgataccctcaaccgcgagggctgtaaggagtatgacgtagctccacaggtcggccaccgcttctgcaaggactttccaggcttcatcccgagcctgctcggggatctcctggaggagaggcagaagataaagaggaagatgaaggcaacaattgacccgatcgagagaaagctccttgattacaggcaacgggccatcaagatccttctaaatagtttttacggctactacggctacgcaagggctcgctggtactgcaaggagtgtgccgagagcgttacggcatggggaagggaatatatcaccatgacaatcagggaaatagaagagaagtatggctttaaagtactttatgcggacactgacggcttcttcgcgacgattcccggggaagatgccgagaccatcaaaaagagggcgatggagttcctcaagtacataaacgccaaactccccggtgcgctcgaacttgagtacgaggacttctacaggcgcggcttcttcgtcaccaagaagaaatacgcggttatcgacgaggagggcaagataacaacgcgcgggctggagatcgtcaggcgcgactggagcgagatagccaaggagacgcaggcgcgggttctggaggcccttctgaaggacggtgacgtcgaagaggccgtgagcatagtcaaagaagtgaccgagaagctgagcaagtacgaggttccgccggagaagctcgttatccacgagcagataacgcgcgagctgaaggactacaaggcaacgggaccacacgtggcgatagcgaagaggttagccgcgagaggcgtcaaaatccgccccgggacagtcatcagctacatcgtgctcaagggctccgggaggataggcgacagggcgattcccttcgacgagttcgaccccacgaagcacaagtacgatgcagagtactacatcgagaaccaggttctacctgccgtcgagaggattctgaaggccttcggctatcgcggtgaggagctcagataccagaagacgaggcaggttggacttggggcgtggctgaagccgaaggggaaggggtga

SEQ ID NO: 6 - protein, 775 aa, Thermococcus siculi
MILDTDYITEDGKPVIRIFKKENGEFKIEYDRTFEPYIYALLKDDSAIEDVKKITAERHGTVVKVKRAEKVQKKFLGRPVEVWKLYFTHPQDVPAIRDKIRKHPAVIDIYEYDIPFAKRYLIDKGLIPMEGEEELKMLAFDIETLYHEGEEFAEGPILMISYADESEARVITWKKIDLPYVDVVSTEKEMIKRFLRVVKEKDPDVLITYNGDNFDFAYLKKRCEKLGINFLLGRDGSEPKIQRMGDRFAVEVKGRIHFDLYPVIRRTINLPTYMLEAVYEAIFGKPKEKVYAEEIATAWETGEGLERVARYSMEDAKVTFELGKEFFPMEAQLSRLVGQSFWDVARSSTGNLVEWFLLRKAYERNELAPNKPSGREYDERRGGYAGGYVKEPEKGLWENIVYLDYKSLYPSIIITHNVSPDTLNREGCKEYDVAPQVGHRFCKDFPGFIPSLLGDLLEERQKIKRKMKATIDPIERKLLDYRQRAIKILLNSFYGYYGYARARWYCKECAESVTAWGREYITMTIREIEEKYGFKVLYADTDGFFATIPGEDAETIKKRAMEFLKYINAKLPGALELEYEDFYRRGFFVTKKKYAVIDEEGKITTRGLEIVRRDWSEIAKETQARVLEALLKDGDVEEAVSIVKEVTEKLSKYEVPPEKLVIHEQITRELKDYKATGPHVAIAKRLAARGVKIRPGTVISYIVLKGSGRIGDRAIPFDEFDPTKHKYDAEYYIENQVLPAVERILKAFGYRGEELRYQKTRQVGLGAWLKPKGKG

SEQ ID NO: 7 - protein, 774 aa, Thermococcus kodakarensis
MILDTDYITEDGKPVIRIFKKENGEFKIEYDRTFEPYFYALLKDDSAIEEVKKITAERHGTVVTVKRVEKVQKKFLGRPVEVWKLYFTHPQDVPAIRDKIREHPAVIDIYEYDIPFAKRYLIDKGLVPMEGDEELKMLAFDIETLYEEGEEFAEGPILMISYADEEGARVITWKNVDLPYVDVVSTEREMIKRFLRVVKEKDPDVLITYNGDNFDFAYLKKRCEKLGINFALGRDGSEPKIQRMGDRFAVEVKGRIHFDLYPVIRRTINLPTYTLEAVYEAVFGQPKEKVYAEEITTAWETGENLERVARYSMEDAKVTYELGKEFLPMEAQLSRLIGQSLWDVSRSSTGNLVEWFLLRKAYERNELAPNKPDEKELARRRQSYEGGYVKEPERGLWENIVYLDFRSLYPSIIITHNVSPDTLNREGCKEYDVAPQVGHRFCKDFPGFIPSLLGDLLEERQKIKKKMKATIDPIERKLLDYRQRAIKILANSYYGYYGYARARWYCKECAESVTAWGREYITMTIKEIEEKYGFKVIYSDTDGFFATIPGADAETVKKKAMEFLKYINAKLPGALELEYEGFYERGFFVTKKKYAVIDEEGKITTRGLEIVRRDWSEIAKETQARVLEALLKDGDVEKAVRIVKEVTEKLSKYEVPPEKLVIHEQITRDLKDYKATGPHVAVAKRLAARGVKIRPGTVISYIVLKGSGRIGDRAIPFDEFDPTKHKYDAEYYIENQVLPAVERILRAFGYRKEDLRYQKTRQVGLSAWLKPKGT

SEQ ID NO: 8 - DNA, 13 bp, Artificial Sequence
  Sample tag sequence
tagaattgaagaa

SEQ ID NO: 9 - DNA, 13 bp, Artificial Sequence
  Sample tag sequence
tggccatagctac

SEQ ID NO: 10 - DNA, 13 bp, Artificial Sequence
  Sample tag sequence
gtcatctgcgacc

SEQ ID NO: 11 - DNA, 13 bp, Artificial Sequence
  Sample tag sequence
ttcgcgcttggac

SEQ ID NO: 12 - DNA, 13 bp, Artificial Sequence
  Sample tag sequence
cgcgaaccgttag

SEQ ID NO: 13 - DNA, 13 bp, Artificial Sequence
  Sample tag sequence
ttgcagcctctaa

SEQ ID NO: 14 - DNA, 13 bp, Artificial Sequence
  Sample tag sequence
tctactagtacga

SEQ ID NO: 15 - DNA, 13 bp, Artificial Sequence
  Sample tag sequence
gtaggttctactg

SEQ ID NO: 16 - DNA, 13 bp, Artificial Sequence
  Sample tag sequence
gccaatatcaagt

SEQ ID NO: 17 - DNA, 13 bp, Artificial Sequence
  Sample tag sequence
ctatcttgctggt

SEQ ID NO: 18 - DNA, 13 bp, Artificial Sequence
  Sample tag sequence
gttctcataggta

SEQ ID NO: 19 - DNA, 13 bp, Artificial Sequence
  Sample tag sequence
gtctatgaaccaa

SEQ ID NO: 20 - DNA, 13 bp, Artificial Sequence
  Sample tag sequence
cggagcgcttatt

SEQ ID NO: 21 - DNA, 13 bp, Artificial Sequence
  Sample tag sequence
tatgccatgagga

SEQ ID NO: 22 - DNA, 13 bp, Artificial Sequence
  Sample tag sequence
atacgactcggag

SEQ ID NO: 23 - DNA, 13 bp, Artificial Sequence
  Sample tag sequence
gatggaactcagc

SEQ ID NO: 24 - DNA, 13 bp, Artificial Sequence
  Sample tag sequence
ggacctgcatgaa

SEQ ID NO: 25 - DNA, 13 bp, Artificial Sequence
  Sample tag sequence
tagactggaactt

SEQ ID NO: 26 - DNA, 13 bp, Artificial Sequence
  Sample tag sequence
gaattacctcgtt

SEQ ID NO: 27 - DNA, 13 bp, Artificial Sequence
  Sample tag sequence
aggatcaggctac

SEQ ID NO: 28 - DNA, 13 bp, Artificial Sequence
  Sample tag sequence
acgcgtagaagag

SEQ ID NO: 29 - DNA, 13 bp, Artificial Sequence
  Sample tag sequence
cttcgagacttac

SEQ ID NO: 30 - DNA, 13 bp, Artificial Sequence
  Sample tag sequence
gacggctaactcc

SEQ ID NO: 31 - DNA, 13 bp, Artificial Sequence
  Sample tag sequence
ttagcattctctt

SEQ ID NO: 32 - DNA, 13 bp, Artificial Sequence
  Sample tag sequence
gcaaggcatagta

SEQ ID NO: 33 - DNA, 13 bp, Artificial Sequence
  Sample tag sequence
acctagatatgga

SEQ ID NO: 34 - DNA, 13 bp, Artificial Sequence
  Sample tag sequence
acgccaaggcgta

SEQ ID NO: 35 - DNA, 13 bp, Artificial Sequence
  Sample tag sequence
tatgacggatccg

SEQ ID NO: 36 - DNA, 13 bp, Artificial Sequence
  Sample tag sequence
cctccattagaga

SEQ ID NO: 37 - DNA, 13 bp, Artificial Sequence
  Sample tag sequence
attgaatactctg

SEQ ID NO: 38 - DNA, 13 bp, Artificial Sequence
  Sample tag sequence
gagatgagaagaa

SEQ ID NO: 39 - DNA, 13 bp, Artificial Sequence
  Sample tag sequence
tctgagtagccgg

SEQ ID NO: 40 - DNA, 13 bp, Artificial Sequence
  Sample tag sequence
aataggtagtacg

SEQ ID NO: 41 - DNA, 13 bp, Artificial Sequence
  Sample tag sequence
gtcgaagaagtcc

SEQ ID NO: 42 - DNA, 13 bp, Artificial Sequence
  Sample tag sequence
tactgcatctcgt

SEQ ID NO: 43 - DNA, 13 bp, Artificial Sequence
  Sample tag sequence
gacgtattagagc

SEQ ID NO: 44 - DNA, 13 bp, Artificial Sequence
  Sample tag sequence
cctgcattattcg

SEQ ID NO: 45 - DNA, 13 bp, Artificial Sequence
  Sample tag sequence
acgaatgatgctc

SEQ ID NO: 46 - DNA, 13 bp, Artificial Sequence
  Sample tag sequence
tactagcagagat

SEQ ID NO: 47 - DNA, 13 bp, Artificial Sequence
  Sample tag sequence
ctcctcatcttcc

SEQ ID NO: 48 - DNA, 13 bp, Artificial Sequence
  Sample tag sequence
tcctctgcgctgc

SEQ ID NO: 49 - DNA, 13 bp, Artificial Sequence
  Sample tag sequence
ccttctcagtccg

SEQ ID NO: 50 - DNA, 13 bp, Artificial Sequence
  Sample tag sequence
cagcttcatagcg

SEQ ID NO: 51 - DNA, 13 bp, Artificial Sequence
  Sample tag sequence
ttgactctcgcgc

SEQ ID NO: 52 - DNA, 13 bp, Artificial Sequence
  Sample tag sequence
tatcctgagcgat

SEQ ID NO: 53 - DNA, 13 bp, Artificial Sequence
  Sample tag sequence
aacgcctagccga

SEQ ID NO: 54 - DNA, 13 bp, Artificial Sequence
  Sample tag sequence
ccgaagacgtcat

SEQ ID NO: 55 - DNA, 13 bp, Artificial Sequence
  Sample tag sequence
gagttctccagat

SEQ ID NO: 56 - DNA, 13 bp, Artificial Sequence
  Sample tag sequence
tgcatccgcgctt

SEQ ID NO: 57 - DNA, 13 bp, Artificial Sequence
  Sample tag sequence
cctgaactcaagt

SEQ ID NO: 58 - DNA, 13 bp, Artificial Sequence
  Sample tag sequence
ggtcgtatgcgta

SEQ ID NO: 59 - DNA, 13 bp, Artificial Sequence
  Sample tag sequence
aggcctctctacc

SEQ ID NO: 60 - DNA, 13 bp, Artificial Sequence
  Sample tag sequence
gtactccatccaa

SEQ ID NO: 61 - DNA, 13 bp, Artificial Sequence
  Sample tag sequence
cagcggacgcgct

SEQ ID NO: 62 - DNA, 13 bp, Artificial Sequence
  Sample tag sequence
atctctcttagca

SEQ ID NO: 63 - DNA, 13 bp, Artificial Sequence
  Sample tag sequence
aagcaataataat

SEQ ID NO: 64 - DNA, 13 bp, Artificial Sequence
  Sample tag sequence
aaggcgactccga

SEQ ID NO: 65 - DNA, 13 bp, Artificial Sequence
  Sample tag sequence
acgtctctaggag

SEQ ID NO: 66 - DNA, 13 bp, Artificial Sequence
  Sample tag sequence
ccatcagacctct

SEQ ID NO: 67 - DNA, 13 bp, Artificial Sequence
  Sample tag sequence
acttaatcgtact

SEQ ID NO: 68 - DNA, 13 bp, Artificial Sequence
  Sample tag sequence
tggaattctccaa

SEQ ID NO: 69 - DNA, 13 bp, Artificial Sequence
  Sample tag sequence
ccatacgatcagg

SEQ ID NO: 70 - DNA, 13 bp, Artificial Sequence
  Sample tag sequence
ttatggagcaata

SEQ ID NO: 71 - DNA, 13 bp, Artificial Sequence
  Sample tag sequence
gctcggcgttcga

SEQ ID NO: 72 - DNA, 13 bp, Artificial Sequence
  Sample tag sequence
ttggccagtcgct

SEQ ID NO: 73 - DNA, 13 bp, Artificial Sequence
  Sample tag sequence
cagatacgtagag

SEQ ID NO: 74 - DNA, 13 bp, Artificial Sequence
  Sample tag sequence
aatgctattatcc

SEQ ID NO: 75 - DNA, 13 bp, Artificial Sequence
  Sample tag sequence
gcagcatgccgat

SEQ ID NO: 76 - DNA, 13 bp, Artificial Sequence
  Sample tag sequence
ggagagttacctc

SEQ ID NO: 77 - DNA, 13 bp, Artificial Sequence
  Sample tag sequence
gagagtccatgat

SEQ ID NO: 78 - DNA, 13 bp, Artificial Sequence
  Sample tag sequence
caatctattctga

SEQ ID NO: 79 - DNA, 13 bp, Artificial Sequence
  Sample tag sequence
gctcttagtatcc

SEQ ID NO: 80 - DNA, 13 bp, Artificial Sequence
  Sample tag sequence
ccatagttatggt

SEQ ID NO: 81 - DNA, 13 bp, Artificial Sequence
  Sample tag sequence
tgcgagatcgaag

SEQ ID NO: 82 - DNA, 13 bp, Artificial Sequence
  Sample tag sequence
agagaagtcgagt

SEQ ID NO: 83 - DNA, 13 bp, Artificial Sequence
  Sample tag sequence
ggtaactccatat

SEQ ID NO: 84 - DNA, 13 bp, Artificial Sequence
  Sample tag sequence
tgctattccaggc

SEQ ID NO: 85 - DNA, 13 bp, Artificial Sequence
  Sample tag sequence
aaccgcgaggctc

SEQ ID NO: 86 - DNA, 13 bp, Artificial Sequence
  Sample tag sequence
ttctagagatacc

SEQ ID NO: 87 - DNA, 13 bp, Artificial Sequence
  Sample tag sequence
ttcgctcaagtat

SEQ ID NO: 88 - DNA, 13 bp, Artificial Sequence
  Sample tag sequence
cagagaaggcgca

SEQ ID NO: 89 - DNA, 13 bp, Artificial Sequence
  Sample tag sequence
tagaattggcctc

SEQ ID NO: 90 - DNA, 13 bp, Artificial Sequence
  Sample tag sequence
ggccattctccag

SEQ ID NO: 91 - DNA, 13 bp, Artificial Sequence
  Sample tag sequence
tccaacgcgcgtt

SEQ ID NO: 92 - DNA, 13 bp, Artificial Sequence
  Sample tag sequence
gccgcagattacg

SEQ ID NO: 93 - DNA, 13 bp, Artificial Sequence
  Sample tag sequence
gcagttcgaacgc

SEQ ID NO: 94 - DNA, 13 bp, Artificial Sequence
  Sample tag sequence
ttctctctgcagg

SEQ ID NO: 95 - DNA, 13 bp, Artificial Sequence
  Sample tag sequence
taagctaccagcg

SEQ ID NO: 96 - DNA, 13 bp, Artificial Sequence
  Sample tag sequence
ctgcatgaggttg

SEQ ID NO: 97 - DNA, 13 bp, Artificial Sequence
  Sample tag sequence
ttgcctagcgagg

SEQ ID NO: 98 - DNA, 13 bp, Artificial Sequence
  Sample tag sequence
caactgaattagg

SEQ ID NO: 99 - DNA, 13 bp, Artificial Sequence
  Sample tag sequence
aagcggtcctctt

SEQ ID NO: 100 - DNA, 13 bp, Artificial Sequence
  Sample tag sequence
aatggaaggaccg

SEQ ID NO: 101 - DNA, 13 bp, Artificial Sequence
  Sample tag sequence
gagttagtaagtt

SEQ ID NO: 102 - DNA, 13 bp, Artificial Sequence
  Sample tag sequence
ttcctaattccaa

SEQ ID NO: 103 - DNA, 13 bp, Artificial Sequence
  Sample tag sequence
gttctggttcgct

SEQ ID NO: 104 - DNA, 13 bp, Artificial Sequence
  Sample tag sequence
gttcatctcttcc

SEQ ID NO: 105 - DNA, 13 bp, Artificial Sequence
  Sample tag sequence
attccgaggaaga

SEQ ID NO: 106 - DNA, 13 bp, Artificial Sequence
  Sample tag sequence
cttagccgagaga

SEQ ID NO: 107 - DNA, 13 bp, Artificial Sequence
  Sample tag sequence
gtctgctacgctt

SEQ ID NO: 108 - DNA, 13 bp, Artificial Sequence
  Sample tag sequence
atggcgccgcgca

SEQ ID NO: 109 - DNA, 13 bp, Artificial Sequence
  Sample tag sequence
taattggttatct

SEQ ID NO: 110 - DNA, 13 bp, Artificial Sequence
  Sample tag sequence
tcggttataagtc

SEQ ID NO: 111 - DNA, 13 bp, Artificial Sequence
  Sample tag sequence
tgcctgagaacgt

SEQ ID NO: 112 - DNA, 13 bp, Artificial Sequence
  Sample tag sequence
agatgcggttaac

SEQ ID NO: 113 - DNA, 13 bp, Artificial Sequence
  Sample tag sequence
atggaataggcga

SEQ ID NO: 114 - DNA, 13 bp, Artificial Sequence
  Sample tag sequence
agagatgcgatcg

SEQ ID NO: 115 - DNA, 13 bp, Artificial Sequence
  Sample tag sequence
ctccaactaacgt

SEQ ID NO: 116 - DNA, 13 bp, Artificial Sequence
  Sample tag sequence
gccttgctactgg

SEQ ID NO: 117 - DNA, 13 bp, Artificial Sequence
  Sample tag sequence
cttcgtctctacg

SEQ ID NO: 118 - DNA, 13 bp, Artificial Sequence
  Sample tag sequence
acgctcatagcct

SEQ ID NO: 119 - DNA, 13 bp, Artificial Sequence
  Sample tag sequence
gtcgaagataagg

SEQ ID NO: 120 - DNA, 13 bp, Artificial Sequence
  Sample tag sequence
gccggagtcctcg

SEQ ID NO: 121 - DNA, 13 bp, Artificial Sequence
  Sample tag sequence
tatacggcgacct

SEQ ID NO: 122 - DNA, 13 bp, Artificial Sequence
  Sample tag sequence
aggtagatattcg

SEQ ID NO: 123 - DNA, 13 bp, Artificial Sequence
  Sample tag sequence
ttaaggtactgct

SEQ ID NO: 124 - DNA, 13 bp, Artificial Sequence
  Sample tag sequence
cggatctggtata

SEQ ID NO: 125 - DNA, 13 bp, Artificial Sequence
  Sample tag sequence
gaggtctcggagg

SEQ ID NO: 126 - DNA, 13 bp, Artificial Sequence
  Sample tag sequence
ggcatcgatggac

SEQ ID NO: 127 - DNA, 13 bp, Artificial Sequence
  Sample tag sequence
gatctccgatata

SEQ ID NO: 128 - DNA, 13 bp, Artificial Sequence
  Sample tag sequence
gattcggaatact

SEQ ID NO: 129 - DNA, 13 bp, Artificial Sequence
  Sample tag sequence
ctgcgatccggcc

SEQ ID NO: 130 - DNA, 13 bp, Artificial Sequence
  Sample tag sequence
gatccggttgcaa

SEQ ID NO: 131 - DNA, 13 bp, Artificial Sequence
  Sample tag sequence
cgtcaggcttgac

SEQ ID NO: 132 - DNA, 13 bp, Artificial Sequence
  Sample tag sequence
tcggcaaggcgag

SEQ ID NO: 133 - DNA, 13 bp, Artificial Sequence
  Sample tag sequence
gaacggcgaacgc

SEQ ID NO: 134 - DNA, 13 bp, Artificial Sequence
  Sample tag sequence
cctcaagcggact

SEQ ID NO: 135 - DNA, 13 bp, Artificial Sequence
  Sample tag sequence
gaagccagatggt

SEQ ID NO: 136 - DNA, 13 bp, Artificial Sequence
  Sample tag sequence
tgctcataccaat

SEQ ID NO: 137 - DNA, 51 bp, Artificial Sequence
  i7 custom index primer (Table 2)
  misc_feature (25)..(36): n is a, c, g or t
caagcagaagacggcatacgagatnnnnnnnnnnnngtctcgtgggctcgg

SEQ ID NO: 138 - DNA, 55 bp, Artificial Sequence
  i5 custom index primer (Table 2)
  misc_feature (30)..(41): n is a, c, g, or t
aatgatacggcgaccaccgagatctacacnnnnnnnnnnnntcgtcggcagcgtc

SEQ ID NO: 139 - DNA, 21 bp, Artificial Sequence
  i7 flow cell primer (Table 3)
caagcagaagacggcatacga

SEQ ID NO: 140 - DNA, 20 bp, Artificial Sequence
  i5 flow cell primer (Table 3)
aatgatacggcgaccaccga

SEQ ID NO: 141 - DNA, 51 bp, Artificial Sequence
  single_mut primer for mutagenesis (Table 5)
  misc_feature (19)..(34): n is a, c, g, or t
tcggtctgcgcctctagcnnnnnnnnnnnnnnnngtctcgtgggctcggag

SEQ ID NO: 142 - DNA, 42 bp, Artificial Sequence
  single_rec primer for recovery (Table 5)
caagcagaagacggcatacgagattcggtctgcgcctctagc

SEQ ID NO: 143 - DNA, 51 bp, Artificial Sequence
  Morphoseq_index_A1
  misc_feature (19)..(21): n is a, c, g, or t
tcggtctgcgcctctagcnnnctctatcgacgtagtctcgtgggctcggag

SEQ ID NO: 144 - DNA, 51 bp, Artificial Sequence
  Morphoseq_index_A2
  misc_feature (19)..(21): n is a, c, g, or t
tcggtctgcgcctctagcnnntaagtctggtctagtctcgtgggctcggag

SEQ ID NO: 145 - DNA, 51 bp, Artificial Sequence
  Morphoseq_index_A3
  misc_feature (19)..(21): n is a, c, g, or t
tcggtctgcgcctctagcnnnacctgcgtaacctgtctcgtgggctcggag

SEQ ID NO: 146 - DNA, 51 bp, Artificial Sequence
  Morphoseq_index_A4
  misc_feature (19)..(21): n is a, c, g, or t
tcggtctgcgcctctagcnnncgtctctaggatggtctcgtgggctcggag

SEQ ID NO: 147 - DNA, 51 bp, Artificial Sequence
  Morphoseq_index_A5
  misc_feature (19)..(21): n is a, c, g, or t
tcggtctgcgcctctagcnnntcattaggtatatgtctcgtgggctcggag

SEQ ID NO: 148 - DNA, 51 bp, Artificial Sequence
  Morphoseq_index_A6
  misc_feature (19)..(21): n is a, c, g, or t
tcggtctgcgcctctagcnnnaagtattccatgagtctcgtgggctcggag

SEQ ID NO: 149 - DNA, 51 bp, Artificial Sequence
  Morphoseq_index_A7
  misc_feature (19)..(21): n is a, c, g, or t
tcggtctgcgcctctagcnnnttctggtacttcagtctcgtgggctcggag

SEQ ID NO: 150 - DNA, 51 bp, Artificial Sequence
  Morphoseq_index_A8
  misc_feature (19)..(21): n is a, c, g, or t
tcggtctgcgcctctagcnnnatgcctcctgcttgtctcgtgggctcggag

SEQ ID NO: 151 - DNA, 51 bp, Artificial Sequence
  Morphoseq_index_A9
  misc_feature (19)..(21): n is a, c, g, or t
tcggtctgcgcctctagcnnntggtaatacgcctgtctcgtgggctcggag

SEQ ID NO: 152 - DNA, 51 bp, Artificial Sequence
  Morphoseq_index_A10
  misc_feature (19)..(21): n is a, c, g, or t
tcggtctgcgcctctagcnnnactgacgattggtgtctcgtgggctcggag

SEQ ID NO: 153 - DNA, 51 bp, Artificial Sequence
  Morphoseq_index_A11
  misc_feature (19)..(21): n is a, c, g, or t
tcggtctgcgcctctagcnnnttagagtagttgcgtctcgtgggctcggag

SEQ ID NO: 154 - DNA, 51 bp, Artificial Sequence
  Morphoseq_index_A12
  misc_feature (19)..(21): n is a, c, g, or t
tcggtctgcgcctctagcnnnaagccgttgaatagtctcgtgggctcggag

SEQ ID NO: 155 - DNA, 51 bp, Artificial Sequence
  Morphoseq_index_B1
  misc_feature (19)..(21): n is a, c, g, or t
tcggtctgcgcctctagcnnntagcctcgctctcgtctcgtgggctcggag

SEQ ID NO: 156 - DNA, 51 bp, Artificial Sequence
  Morphoseq_index_B2
  misc_feature (19)..(21): n is a, c, g, or t
tcggtctgcgcctctagcnnncttggccttgcaagtctcgtgggctcggag

SEQ ID NO: 157 - DNA, 51 bp, Artificial Sequence
  Morphoseq_index_B3
  misc_feature (19)..(21): n is a, c, g, or t
tcggtctgcgcctctagcnnnctatcttcaactggtctcgtgggctcggag

SEQ ID NO: 158 - DNA, 51 bp, Artificial Sequence
  Morphoseq_index_B4
  misc_feature (19)..(21): n is a, c, g, or t
tcggtctgcgcctctagcnnnatccatacggactgtctcgtgggctcggag

SEQ ID NO: 159 - DNA, 51 bp, Artificial Sequence
  Morphoseq_index_B5
  misc_feature (19)..(21): n is a, c, g, or t
tcggtctgcgcctctagcnnncgctcgctcatatgtctcgtgggctcggag

SEQ ID NO: 160 - DNA, 51 bp, Artificial Sequence
  Morphoseq_index_B6
  misc_feature (19)..(21): n is a, c, g, or t
tcggtctgcgcctctagcnnncgtatcgaattcagtctcgtgggctcggag

SEQ ID NO: 161 - DNA, 51 bp, Artificial Sequence
  Morphoseq_index_B7
  misc_feature (19)..(21): n is a, c, g, or t
tcggtctgcgcctctagcnnnattcttctcggtagtctcgtgggctcggag

SEQ ID NO: 162 - DNA, 51 bp, Artificial Sequence
  Morphoseq_index_B8
  misc_feature (19)..(21): n is a, c, g, or t
tcggtctgcgcctctagcnnncaagttgcagcaggtctcgtgggctcggag

SEQ ID NO: 163 - DNA, 51 bp, Artificial Sequence
  Morphoseq_index_B9
  misc_feature (19)..(21): n is a, c, g, or t
tcggtctgcgcctctagcnnnactaatctggtacgtctcgtgggctcggag

SEQ ID NO: 164 - DNA, 51 bp, Artificial Sequence
  Morphoseq_index_B10
  misc_feature (19)..(21): n is a, c, g, or t
tcggtctgcgcctctagcnnncaggaagattagtgtctcgtgggctcggag

SEQ ID NO: 165 - DNA, 51 bp, Artificial Sequence
  Morphoseq_index_B11
  misc_feature (19)..(21): n is a, c, g, or t
tcggtctgcgcctctagcnnnaataactagcttggtctcgtgggctcggag

SEQ ID NO: 166 - DNA, 51 bp, Artificial Sequence
  Morphoseq_index_B12
  misc_feature (19)..(21): n is a, c, g, or t
tcggtctgcgcctctagcnnntacgacttactaagtctcgtgggctcggag

SEQ ID NO: 167 - DNA, 51 bp, Artificial Sequence
  Morphoseq_index_C1
  misc_feature (19)..(21): n is a, c, g, or t
tcggtctgcgcctctagcnnnctcggcttctcctgtctcgtgggctcggag

SEQ ID NO: 168 - DNA, 51 bp, Artificial Sequence
  Morphoseq_index_C2
  misc_feature (19)..(21): n is a, c, g, or t
tcggtctgcgcctctagcnnnttcctctctatcagtctcgtgggctcggag

SEQ ID NO: 169 - DNA, 51 bp, Artificial Sequence
  Morphoseq_index_C3
  misc_feature (19)..(21): n is a, c, g, or t
tcggtctgcgcctctagcnnnatggattcctagagtctcgtgggctcggag

SEQ ID NO: 170 - DNA, 51 bp, Artificial Sequence
  Morphoseq_index_C4
  misc_feature (19)..(21): n is a, c, g, or t
tcggtctgcgcctctagcnnnttcttgagtaagggtctcgtgggctcggag

SEQ ID NO: 171 - DNA, 51 bp, Artificial Sequence
  Morphoseq_index_C5
  misc_feature (19)..(21): n is a, c, g, or t
tcggtctgcgcctctagcnnnactactacgaagggtctcgtgggctcggag

SEQ ID NO: 172 - DNA, 51 bp, Artificial Sequence
  Morphoseq_index_C6
  misc_feature (19)..(21): n is a, c, g, or t
tcggtctgcgcctctagcnnncatcgctatcgttgtctcgtgggctcggag

SEQ ID NO: 173 - DNA, 51 bp, Artificial Sequence
  Morphoseq_index_C7
  misc_feature (19)..(21): n is a, c, g, or t
tcggtctgcgcctctagcnnnaagttccgcattagtctcgtgggctcggag

SEQ ID NO: 174 - DNA, 51 bp, Artificial Sequence
  Morphoseq_index_C8
  misc_feature (19)..(21): n is a, c, g, or t
tcggtctgcgcctctagcnnnacttaagttgaaggtctcgtgggctcggag

SEQ ID NO: 175 - DNA, 51 bp, Artificial Sequence
  Morphoseq_index_C9
  misc_feature (19)..(21): n is a, c, g, or t
tcggtctgcgcctctagcnnntgagtaattcgacgtctcgtgggctcggag

SEQ ID NO: 176 - DNA, 51 bp, Artificial Sequence
  Morphoseq_index_C10
  misc_feature (19)..(21): n is a, c, g, or t
tcggtctgcgcctctagcnnnagctgaagacttagtctcgtgggctcggag

SEQ ID NO: 177 - DNA, 51 bp, Artificial Sequence
  Morphoseq_index_C11
  misc_feature (19)..(21): n is a, c, g, or t
tcggtctgcgcctctagcnnncaaggatagaattgtctcgtgggctcggag

SEQ ID NO: 178 - DNA, 51 bp, Artificial Sequence
  Morphoseq_index_C12
  misc_feature (19)..(21): n is a, c, g, or t
tcggtctgcgcctctagcnnnagcatgattgcgggtctcgtgggctcggag

SEQ ID NO: 179 - DNA, 51 bp, Artificial Sequence
  Morphoseq_index_D1
  misc_feature (19)..(21): n is a, c, g, or t
tcggtctgcgcctctagcnnnacctgaagctgctgtctcgtgggctcggag

SEQ ID NO: 180 - DNA, 51 bp, Artificial Sequence
  Morphoseq_index_D2
  misc_feature (19)..(21): n is a, c, g, or t
tcggtctgcgcctctagcnnncatatggtaacgtgtctcgtgggctcggag

SEQ ID NO: 181 - DNA, 51 bp, Artificial Sequence
  Morphoseq_index_D3
  misc_feature (19)..(21): n is a, c, g, or t
tcggtctgcgcctctagcnnnatggaatacgcgggtctcgtgggctcggag

SEQ ID NO: 182 - DNA, 51 bp, Artificial Sequence
  Morphoseq_index_D4
  misc_feature (19)..(21): n is a, c, g, or t
tcggtctgcgcctctagcnnntctattactctcagtctcgtgggctcggag

SEQ ID NO: 183 - DNA, 51 bp, Artificial Sequence
  Morphoseq_index_D5
  misc_feature (19)..(21): n is a, c, g, or t
tcggtctgcgcctctagcnnntcgattactcaaggtctcgtgggctcggag

SEQ ID NO: 184 - DNA, 51 bp, Artificial Sequence
  Morphoseq_index_D6
  misc_feature (19)..(21): n is a, c, g, or t
tcggtctgcgcctctagcnnnctgcttatattcagtctcgtgggctcggag

SEQ ID NO: 185 - DNA, 51 bp, Artificial Sequence
  Morphoseq_index_D7
  misc_feature (19)..(21): n is a, c, g, or t
tcggtctgcgcctctagcnnntatgccatctagtgtctcgtgggctcggag

SEQ ID NO: 186 - DNA, 51 bp, Artificial Sequence
  Morphoseq_index_D8
  misc_feature (19)..(21): n is a, c, g, or t
tcggtctgcgcctctagcnnnaatgcttgaatgggtctcgtgggctcggag

SEQ ID NO: 187 - DNA, 51 bp, Artificial Sequence
  Morphoseq_index_D9
  misc_feature (19)..(21): n is a, c, g, or t
tcggtctgcgcctctagcnnnacgttcaggagatgtctcgtgggctcggag

SEQ ID NO: 188 - DNA, 51 bp, Artificial Sequence
  Morphoseq_index_D10
  misc_feature (19)..(21): n is a, c, g, or t
tcggtctgcgcctctagcnnntcttcctagcttagtctcgtgggctcggag

SEQ ID NO: 189 - DNA, 51 bp, Artificial Sequence
  Morphoseq_index_D11
  misc_feature (19)..(21): n is a, c, g, or t
tcggtctgcgcctctagcnnnaagtcggatcatggtctcgtgggctcggag

SEQ ID NO: 190 - DNA, 51 bp, Artificial Sequence
  Morphoseq_index_D12
  misc_feature (19)..(21): n is a, c, g, or t
tcggtctgcgcctctagcnnncagaaccggaagagtctcgtgggctcggag

SEQ ID NO: 191 - DNA, 51 bp, Artificial Sequence
  Morphoseq_index_E1
  misc_feature (19)..(21): n is a, c, g, or t
tcggtctgcgcctctagcnnnatgctggctctcggtctcgtgggctcggag

SEQ ID NO: 192 - DNA, 51 bp, Artificial Sequence
  Morphoseq_index_E2
  misc_feature (19)..(21): n is a, c, g, or t
tcggtctgcgcctctagcnnntggcctgatgaacgtctcgtgggctcggag

SEQ ID NO: 193 - DNA, 51 bp, Artificial Sequence
  Morphoseq_index_E3
  misc_feature (19)..(21): n is a, c, g, or t
tcggtctgcgcctctagcnnnaatggacgccaaggtctcgtgggctcggag

SEQ ID NO: 194 - DNA, 51 bp, Artificial Sequence
  Morphoseq_index_E4
  misc_feature (19)..(21): n is a, c, g, or t
tcggtctgcgcctctagcnnnctcaactggacctgtctcgtgggctcggag

SEQ ID NO: 195 - DNA, 51 bp, Artificial Sequence
  Morphoseq_index_E5
  misc_feature (19)..(21): n is a, c, g, or t
tcggtctgcgcctctagcnnnaattcatcgtctggtctcgtgggctcggag

SEQ ID NO: 196 - DNA, 51 bp, Artificial Sequence
  Morphoseq_index_E6
  misc_feature (19)..(21): n is a, c, g, or t
tcggtctgcgcctctagcnnntcggactaaggtagtctcgtgggctcggag

SEQ ID NO: 197 - DNA, 51 bp, Artificial Sequence
  Morphoseq_index_E7
  misc_feature (19)..(21): n is a, c, g, or t
tcggtctgcgcctctagcnnncgaagctcctccagtctcgtgggctcggag

SEQ ID NO: 198 - DNA, 51 bp, Artificial Sequence
  Morphoseq_index_E8
  misc_feature (19)..(21): n is a, c, g, or t
tcggtctgcgcctctagcnnntgccatagatagcgtctcgtgggctcggag

SEQ ID NO: 199 - DNA, 51 bp, Artificial Sequence
  Morphoseq_index_E9
  misc_feature (19)..(21): n is a, c, g, or t
tcggtctgcgcctctagcnnntaactctcggtatgtctcgtgggctcggag

SEQ ID NO: 200 - DNA, 51 bp, Artificial Sequence
  Morphoseq_index_E10
  misc_feature (19)..(21): n is a, c, g, or t
tcggtctgcgcctctagcnnnaattctggatctcgtctcgtgggctcggag

SEQ ID NO: 201 - DNA, 51 bp, Artificial Sequence
  Morphoseq_index_E11
  misc_feature (19)..(21): n is a, c, g, or t
tcggtctgcgcctctagcnnnattgaagagagtcgtctcgtgggctcggag

SEQ ID NO: 202 - DNA, 51 bp, Artificial Sequence
  Morphoseq_index_E12
  misc_feature (19)..(21): n is a, c, g, or t
tcggtctgcgcctctagcnnntcataggttctgagtctcgtgggctcggag

SEQ ID NO: 203 - DNA, 51 bp, Artificial Sequence
  Morphoseq_index_F1
  misc_feature (19)..(21): n is a, c, g, or t
tcggtctgcgcctctagcnnnatcatagtattatgtctcgtgggctcggag

SEQ ID NO: 204 - DNA, 51 bp, Artificial Sequence
  Morphoseq_index_F2
  misc_feature (19)..(21): n is a, c, g, or t
tcggtctgcgcctctagcnnncgctggattcggtgtctcgtgggctcggag

SEQ ID NO: 205 - DNA, 51 bp, Artificial Sequence
  Morphoseq_index_F3
  misc_feature (19)..(21): n is a, c, g, or t
tcggtctgcgcctctagcnnnttagcggaatggagtctcgtgggctcggag

SEQ ID NO: 206 - DNA, 51 bp, Artificial Sequence
  Morphoseq_index_F4
  misc_feature (19)..(21): n is a, c, g, or t
tcggtctgcgcctctagcnnnaagaagtcgtctggtctcgtgggctcggag

SEQ ID NO: 207 - DNA, 51 bp, Artificial Sequence
  Morphoseq_index_F5
  misc_feature (19)..(21): n is a, c, g, or t
tcggtctgcgcctctagcnnnaagaaggagttacgtctcgtgggctcggag

SEQ ID NO: 208 - DNA, 51 bp, Artificial Sequence
  Morphoseq_index_F6
  misc_feature (19)..(21): n is a, c, g, or t
tcggtctgcgcctctagcnnncgctctcgtcagggtctcgtgggctcggag

SEQ ID NO: 209 - DNA, 51 bp, Artificial Sequence
  Morphoseq_index_F7
  misc_feature (19)..(21): n is a, c, g, or t
tcggtctgcgcctctagcnnnaccgcgttctcttgtctcgtgggctcggag

SEQ ID NO: 210 - DNA, 51 bp, Artificial Sequence
  Morphoseq_index_F8
  misc_feature (19)..(21): n is a, c, g, or t
tcggtctgcgcctctagcnnntccagaagaagaagtctcgtgggctcggag

SEQ ID NO: 211 - DNA, 51 bp, Artificial Sequence
  Morphoseq_index_F9
  misc_feature (19)..(21): n is a, c, g, or t
tcggtctgcgcctctagcnnntcttcggtccaacgtctcgtgggctcggag

SEQ ID NO: 212 - DNA, 51 bp, Artificial Sequence
  Morphoseq_index_F10
  misc_feature (19)..(21): n is a, c, g, or t
tcggtctgcgcctctagcnnnatatgccaataacgtctcgtgggctcggag

SEQ ID NO: 213 - DNA, 51 bp, Artificial Sequence
  Morphoseq_index_F11
  misc_feature (19)..(21): n is a, c, g, or t
tcggtctgcgcctctagcnnntctatcgtaagtcgtctcgtgggctcggag

SEQ ID NO: 214 - DNA, 51 bp, Artificial Sequence
  Morphoseq_index_F12
  misc_feature (19)..(21): n is a, c, g, or t
tcggtctgcgcctctagcnnntgctaaggtcttcgtctcgtgggctcggag

SEQ ID NO: 215 - DNA, 51 bp, Artificial Sequence
  Morphoseq_index_G1
  misc_feature (19)..(21): n is a, c, g, or t
tcggtctgcgcctctagcnnnaggaccaaggctcgtctcgtgggctcggag

SEQ ID NO: 216 - DNA, 51 bp, Artificial Sequence
  Morphoseq_index_G2
  misc_feature (19)..(21): n is a, c, g, or t
tcggtctgcgcctctagcnnntcaacgtcatgctgtctcgtgggctcggag

SEQ ID NO: 217 - DNA, 51 bp, Artificial Sequence
  Morphoseq_index_G3
  misc_feature (19)..(21): n is a, c, g, or t
tcggtctgcgcctctagcnnnttcaaggatcaaggtctcgtgggctcggag

SEQ ID NO: 218 - DNA, 51 bp, Artificial Sequence
  Morphoseq_index_G4
  misc_feature (19)..(21): n is a, c, g, or t
tcggtctgcgcctctagcnnnacggtactgcttagtctcgtgggctcggag

SEQ ID NO: 219 - DNA, 51 bp, Artificial Sequence
  Morphoseq_index_G5
  misc_feature (19)..(21): n is a, c, g, or t
tcggtctgcgcctctagcnnnttcgaaccatccggtctcgtgggctcggag

SEQ ID NO: 220 - DNA, 51 bp, Artificial Sequence
  Morphoseq_index_G6
  misc_feature (19)..(21): n is a, c, g, or t
tcggtctgcgcctctagcnnntggatgcatgaacgtctcgtgggctcggag

SEQ ID NO: 221 - DNA, 51 bp, Artificial Sequence
  Morphoseq_index_G7
  misc_feature (19)..(21): n is a, c, g, or t
tcggtctgcgcctctagcnnnctcagaaggtactgtctcgtgggctcggag

SEQ ID NO: 222 - DNA, 51 bp, Artificial Sequence
  Morphoseq_index_G8
  misc_feature (19)..(21): n is a, c, g, or t
tcggtctgcgcctctagcnnntggacggccttgcgtctcgtgggctcggag

SEQ ID NO: 223 - DNA, 51 bp, Artificial Sequence
  Morphoseq_index_G9
  misc_feature (19)..(21): n is a, c, g, or t
tcggtctgcgcctctagcnnnaatcgtatagcaagtctcgtgggctcggag

SEQ ID NO: 224 - DNA, 51 bp, Artificial Sequence
  Morphoseq_index_G10
  misc_feature (19)..(21): n is a, c, g, or t
tcggtctgcgcctctagcnnntacggcaagctatgtctcgtgggctcggag

SEQ ID NO: 225 - DNA, 51 bp, Artificial Sequence
  Morphoseq_index_G11
  misc_feature (19)..(21): n is a, c, g, or t
tcggtctgcgcctctagcnnncaaccaaggaagcgtctcgtgggctcggag

SEQ ID NO: 226 - DNA, 51 bp, Artificial Sequence
  Morphoseq_index_G12
  misc_feature (19)..(21): n is a, c, g, or t
tcggtctgcgcctctagcnnntgcgaataatgcggtctcgtgggctcggag

SEQ ID NO: 227 - DNA, 51 bp, Artificial Sequence
  Morphoseq_index_H1
  misc_feature (19)..(21): n is a, c, g, or t
tcggtctgcgcctctagcnnnatctcttaagaatgtctcgtgggctcggag

SEQ ID NO: 228 - DNA, 51 bp, Artificial Sequence
  Morphoseq_index_H2
  misc_feature (19)..(21): n is a, c, g, or t
tcggtctgcgcctctagcnnnaagatatgattaagtctcgtgggctcggag

SEQ ID NO: 229 - DNA, 51 bp, Artificial Sequence
  Morphoseq_index_H3
  misc_feature (19)..(21): n is a, c, g, or t
tcggtctgcgcctctagcnnnatctcaataataagtctcgtgggctcggag

SEQ ID NO: 230 - DNA, 51 bp, Artificial Sequence
  Morphoseq_index_H4
  misc_feature (19)..(21): n is a, c, g, or t
tcggtctgcgcctctagcnnnctgcatctatggagtctcgtgggctcggag

SEQ ID NO: 231 - DNA, 51 bp, Artificial Sequence
  Morphoseq_index_H5
  misc_feature (19)..(21): n is a, c, g, or t
tcggtctgcgcctctagcnnnaggagtcttagcagtctcgtgggctcggag

SEQ ID NO: 232 - DNA, 51 bp, Artificial Sequence
  Morphoseq_index_H6
  misc_feature (19)..(21): n is a, c, g, or t
tcggtctgcgcctctagcnnnaataggactctgcgtctcgtgggctcggag

SEQ ID NO: 233 - DNA, 51 bp, Artificial Sequence
  Morphoseq_index_H7
  misc_feature (19)..(21): n is a, c, g, or t
tcggtctgcgcctctagcnnntcttacgttgccggtctcgtgggctcggag

SEQ ID NO: 234 - DNA, 51 bp, Artificial Sequence
  Morphoseq_index_H8
  misc_feature (19)..(21): n is a, c, g, or t
tcggtctgcgcctctagcnnntggcatgaagtatgtctcgtgggctcggag

SEQ ID NO: 235 - DNA, 51 bp, Artificial Sequence
  Morphoseq_index_H9
  misc_feature (19)..(21): n is a, c, g, or t
tcggtctgcgcctctagcnnncaatatgccaggtgtctcgtgggctcggag

SEQ ID NO: 236 - DNA, 51 bp, Artificial Sequence
  Morphoseq_index_H10
  misc_feature (19)..(21): n is a, c, g, or t
tcggtctgcgcctctagcnnncataaggaggtaagtctcgtgggctcggag

SEQ ID NO: 237 - DNA, 51 bp, Artificial Sequence
  Morphoseq_index_H11
  misc_feature (19)..(21): n is a, c, g, or t
tcggtctgcgcctctagcnnnacggtaagcaagcgtctcgtgggctcggag

SEQ ID NO: 238 - DNA, 51 bp, Artificial Sequence
  Morphoseq_index_H12
  misc_feature (19)..(21): n is a, c, g, or t
tcggtctgcgcctctagcnnnaactgcttcgatcgtctcgtgggctcggag

SEQ ID NO: 239 - DNA, 42 bp, Artificial Sequence; identical to SEQ ID NO: 142
  Recovery primer

SEQ ID NO: 240 - DNA, 21 bp, Artificial Sequence
  Enrichment primer
caagcagaagacggcatacga

SEQ ID NO: 241 - DNA, 55 bp, Artificial Sequence
  Custom_i5_index_end
  misc_feature (36)..(41): n is a, c, g, or t
aatgatacggcgaccaccgagatctacacaagttcnnnnnntcgtcggcagcgtc

SEQ ID NO: 242 - DNA, 51 bp, Artificial Sequence
  Custom_i7_index_int
  misc_feature (25)..(30): n is a, c, g, or t
caagcagaagacggcatacgagatnnnnnnttaggagtctcgtgggctcgg

SEQ ID NO: 243 - DNA, 55 bp, Artificial Sequence
  Custom_i5_index_int
  misc_feature (36)..(41): n is a, c, g, or t
aatgatacggcgaccaccgagatctacactaaccgnnnnnntcgtcggcagcgtc

SEQ ID NO: 244 - DNA, 51 bp, Artificial Sequence
  Custom_i7_index_1
  misc_feature (25)..(30): n is a, c, g, or t
caagcagaagacggcatacgagatnnnnnnctacctgtctcgtgggctcgg

SEQ ID NO: 245 - DNA, 51 bp, Artificial Sequence
  Custom_i7_index_2
  misc_feature (25)..(30): n is a, c, g, or t
caagcagaagacggcatacgagatnnnnnntctgaagtctcgtgggctcgg

SEQ ID NO: 246 - DNA, 51 bp, Artificial Sequence
  Custom_i7_index_3
  misc_feature (25)..(30): n is a, c, g, or t
caagcagaagacggcatacgagatnnnnnnaatacggtctcgtgggctcgg

SEQ ID NO: 247 - DNA, 51 bp, Artificial Sequence
  Custom_i7_index_4
  misc_feature (25)..(30): n is a, c, g, or t
caagcagaagacggcatacgagatnnnnnnatactcgtctcgtgggctcgg

SEQ ID NO: 248 - DNA, 51 bp, Artificial Sequence
  Custom_i7_index_5
  misc_feature (25)..(30): n is a, c, g, or t
caagcagaagacggcatacgagatnnnnnnaggagcgtctcgtgggctcgg

SEQ ID NO: 249 - DNA, 51 bp, Artificial Sequence
  Custom_i7_index_6
  misc_feature (25)..(30): n is a, c, g, or t
caagcagaagacggcatacgagatnnnnnnaagttcgtctcgtgggctcgg

SEQ ID NO: 250 - DNA, 51 bp, Artificial Sequence
  Custom_i7_index_7
  misc_feature (25)..(30): n is a, c, g, or t
caagcagaagacggcatacgagatnnnnnntatagtgtctcgtgggctcgg

SEQ ID NO: 251 - DNA, 51 bp, Artificial Sequence
  Custom_i7_index_8
  misc_feature (25)..(30): n is a, c, g, or t
caagcagaagacggcatacgagatnnnnnncggaatgtctcgtgggctcgg

SEQ ID NO: 252 - DNA, 51 bp, Artificial Sequence
  Custom_i7_index_9
  misc_feature (25)..(30): n is a, c, g, or t
caagcagaagacggcatacgagatnnnnnnggaacggtctcgtgggctcgg

SEQ ID NO: 253 - DNA, 51 bp, Artificial Sequence
  Custom_i7_index_10
  misc_feature (25)..(30): n is a, c, g, or t
caagcagaagacggcatacgagatnnnnnnggcttggtctcgtgggctcgg

SEQ ID NO: 254 - DNA, 51 bp, Artificial Sequence
  Custom_i7_index_11
  misc_feature (25)..(30): n is a, c, g, or t
caagcagaagacggcatacgagatnnnnnnaggcctgtctcgtgggctcgg

SEQ ID NO: 255 - DNA, 51 bp, Artificial Sequence
  Custom_i7_index_12
  misc_feature (25)..(30): n is a, c, g, or t
caagcagaagacggcatacgagatnnnnnncttgccgtctcgtgggctcgg

SEQ ID NO: 256 - DNA, 51 bp, Artificial Sequence
  Custom_i7_index_13
  misc_feature (25)..(30): n is a, c, g, or t
caagcagaagacggcatacgagatnnnnnntagcgcgtctcgtgggctcgg

SEQ ID NO: 257 - DNA, 51 bp, Artificial Sequence
  Custom_i7_index_14
  misc_feature (25)..(30): n is a, c, g, or t
caagcagaagacggcatacgagatnnnnnngaccgggtctcgtgggctcgg

SEQ ID NO: 258 - DNA, 51 bp, Artificial Sequence
  Custom_i7_index_15
  misc_feature (25)..(30): n is a, c, g, or t
caagcagaagacggcatacgagatnnnnnnccatgagtctcgtgggctcgg

SEQ ID NO: 259 - DNA, 51 bp, Artificial Sequence
  Custom_i7_index_16
  misc_feature (25)..(30): n is a, c, g, or t
caagcagaagacggcatacgagatnnnnnnttggaggtctcgtgggctcgg

SEQ ID NO: 260 - DNA, 51 bp, Artificial Sequence
  Custom_i7_index_17
  misc_feature (25)..(30): n is a, c, g, or t
caagcagaagacggcatacgagatnnnnnngcctgcgtctcgtgggctcgg

SEQ ID NO: 261 - DNA, 51 bp, Artificial Sequence
  Custom_i7_index_18
  misc_feature (25)..(30): n is a, c, g, or t
caagcagaagacggcatacgagatnnnnnnggcaacgtctcgtgggctcgg

SEQ ID NO: 262 - DNA, 51 bp, Artificial Sequence
  Custom_i7_index_19
  misc_feature (25)..(30): n is a, c, g, or t
caagcagaagacggcatacgagatnnnnnntaaccggtctcgtgggctcgg

SEQ ID NO: 263 - DNA, 51 bp, Artificial Sequence
  Custom_i7_index_20
  misc_feature (25)..(30): n is a, c, g, or t
caagcagaagacggcatacgagatnnnnnncgcgaggtctcgtgggctcgg

SEQ ID NO: 264 - DNA, 51 bp, Artificial Sequence
  Custom_i7_index_21
  misc_feature (25)..(30): n is a, c, g, or t
caagcagaagacggcatacgagatnnnnnnaaccatgtctcgtgggctcgg

SEQ ID NO: 265 - DNA, 51 bp, Artificial Sequence
  Custom_i7_index_22
  misc_feature (25)..(30): n is a, c, g, or t
caagcagaagacggcatacgagatnnnnnntcatacgtctcgtgggctcgg

SEQ ID NO: 266 - DNA, 51 bp, Artificial Sequence
  Custom_i7_index_23
  misc_feature (25)..(30): n is a, c, g, or t
caagcagaagacggcatacgagatnnnnnnacggttgtctcgtgggctcgg

SEQ ID NO: 267 - DNA, 51 bp, Artificial Sequence
  Custom_i7_index_24
  misc_feature (25)..(30): n is a, c, g, or t
caagcagaagacggcatacgagatnnnnnnggttctgtctcgtgggctcgg

SEQ ID NO: 268 - DNA, 55 bp, Artificial Sequence
  Custom_i5_index_1
  misc_feature (36)..(41): n is a, c, g, or t
aatgatacggcgaccaccgagatctacacttaggannnnnntcgtcggcagcgtc

SEQ ID NO: 269 - DNA, 55 bp, Artificial Sequence
  Custom_i5_index_2
  misc_feature (36)..(41): n is a, c, g, or t
aatgatacggcgaccaccgagatctacacaggagcnnnnnntcgtcggcagcgtc

SEQ ID NO: 270 - DNA, 55 bp, Artificial Sequence
  Custom_i5_index_3
  misc_feature (36)..(41): n is a, c, g, or t
aatgatacggcgaccaccgagatctacacacggttnnnnnntcgtcggcagcgtc

SEQ ID NO: 271 - DNA, 55 bp, Artificial Sequence
  Custom_i5_index_4
  misc_feature (36)..(41): n is a, c, g, or t
aatgatacggcgaccaccgagatctacacgcctgcnnnnnntcgtcggcagcgtc

SEQ ID NO: 272 - DNA, 55 bp, Artificial Sequence
  Custom_i5_index_5
  misc_feature (36)..(41): n is a, c, g, or t
aatgatacggcgaccaccgagatctacactagcgcnnnnnntcgtcggcagcgtc

SEQ ID NO: 273 - DNA, 55 bp, Artificial Sequence
  Custom_i5_index_6
  misc_feature (36)..(41): n is a, c, g, or t
aatgatacggcgaccaccgagatctacacggttctnnnnnntcgtcggcagcgtc

SEQ ID NO: 274 - DNA, 55 bp, Artificial Sequence
  Custom_i5_index_7
  misc_feature (36)..(41): n is a, c, g, or t
aatgatacggcgaccaccgagatctacacaggcctnnnnnntcgtcggcagcgtc

SEQ ID NO: 275 - DNA, 55 bp, Artificial Sequence
  Custom_i5_index_8
  misc_feature (36)..(41): n is a, c, g, or t
aatgatacggcgaccaccgagatctacaccttgccnnnnnntcgtcggcagcgtc

SEQ ID NO: 276 - DNA, 55 bp, Artificial Sequence
  Custom_i5_index_9
  misc_feature (36)..(41): n is a, c, g, or t
aatgatacggcgaccaccgagatctacacctacctnnnnnntcgtcggcagcgtc

SEQ ID NO: 277 - DNA, 55 bp, Artificial Sequence
  Custom_i5_index_10
  misc_feature (36)..(41): n is a, c, g, or t
aatgatacggcgaccaccgagatctacactcatacnnnnnntcgtcggcagcgtc

SEQ ID NO: 278 - DNA, 55 bp, Artificial Sequence
  Custom_i5_index_11
  misc_feature (36)..(41): n is a, c, g, or t
aatgatacggcgaccaccgagatctacacgtcgcgnnnnnntcgtcggcagcgtc

SEQ ID NO: 279 - DNA, 55 bp, Artificial Sequence
  Custom_i5_index_12
  misc_feature (36)..(41): n is a, c, g, or t
aatgatacggcgaccaccgagatctacacaaccatnnnnnntcgtcggcagcgtc

SEQ ID NO: 280 - DNA, 55 bp, Artificial Sequence
  Custom_i5_index_13
  misc_feature (36)..(41): n is a, c, g, or t
aatgatacggcgaccaccgagatctacacctggtannnnnntcgtcggcagcgtc

SEQ ID NO: 281 - DNA, 55 bp, Artificial Sequence
  Custom_i5_index_14
  misc_feature (36)..(41): n is a, c, g, or t
aatgatacggcgaccaccgagatctacacgaccggnnnnnntcgtcggcagcgtc

SEQ ID NO: 282 - DNA, 55 bp, Artificial Sequence
  Custom_i5_index_15
  misc_feature (36)..(41): n is a, c, g, or t
aatgatacggcgaccaccgagatctacaccggaatnnnnnntcgtcggcagcgtc

SEQ ID NO: 283 - DNA, 55 bp, Artificial Sequence
  Custom_i5_index_16
  misc_feature (36)..(41): n is a, c, g, or t
aatgatacggcgaccaccgagatctacactatagtnnnnnntcgtcggcagcgtc

SEQ ID NO: 284 - DNA, 55 bp, Artificial Sequence
  Custom_i5_index_17
  misc_feature (36)..(41): n is a, c, g, or t
aatgatacggcgaccaccgagatctacaccaatatnnnnnntcgtcggcagcgtc

SEQ ID NO: 285 - DNA, 55 bp, Artificial Sequence
  Custom_i5_index_18
  misc_feature (36)..(41): n is a, c, g, or t
aatgatacggcgaccaccgagatctacacggcttgnnnnnntcgtcggcagcgtc

SEQ ID NO: 286 - DNA, 55 bp, Artificial Sequence
  Custom_i5_index_19
  misc_feature (36)..(41): n is a, c, g, or t
aatgatacggcgaccaccgagatctacacaatacgnnnnnntcgtcggcagcgtc

SEQ ID NO: 287 - DNA, 55 bp, Artificial Sequence
  Custom_i5_index_20
  misc_feature (36)..(41): n is a, c, g, or t
aatgatacggcgaccaccgagatctacacccatgannnnnntcgtcggcagcgtc

SEQ ID NO: 288 - DNA, 55 bp, Artificial Sequence
  Custom_i5_index_21
  misc_feature (36)..(41): n is a, c, g, or t
aatgatacggcgaccaccgagatctacactctgaannnnnntcgtcggcagcgtc

SEQ ID NO: 289 - DNA, 55 bp, Artificial Sequence
  Custom_i5_index_22
  misc_feature (36)..(41): n is a, c, g, or t
aatgatacggcgaccaccgagatctacacggcaacnnnnnntcgtcggcagcgtc

SEQ ID NO: 290 - DNA, 55 bp, Artificial Sequence
  Custom_i5_index_23
  misc_feature (36)..(41): n is a, c, g, or t
aatgatacggcgaccaccgagatctacacatactcnnnnnntcgtcggcagcgtc

SEQ ID NO: 291 - DNA, 55 bp, Artificial Sequence
  Custom_i5_index_24
  misc_feature (36)..(41): n is a, c, g, or t
aatgatacggcgaccaccgagatctacacttggagnnnnnntcgtcggcagcgtc